European Patent Application EP 4 257 610 A1, published October 11, 2023. Title: ROR1-targeting antibody and use thereof. Applicant: Bioheng Therapeutics Limited. The sequence listing filed with the application follows.

SEQUENCE LISTING (95 sequences)

SEQ ID NO: 1 - protein, 11 aa, Artificial Sequence
  CDR-L1
ITSTDIDDDMN

SEQ ID NO: 2 - protein, 7 aa, Artificial Sequence
  CDR-L2
EGNALRP

SEQ ID NO: 3 - protein, 9 aa, Artificial Sequence
  CDR-L3
LQSNKLPLT

SEQ ID NO: 4 - protein, 8 aa, Artificial Sequence
  CDR-H1
GYSITSDY

SEQ ID NO: 5 - protein, 5 aa, Artificial Sequence
  CDR-H2
SYSGY

SEQ ID NO: 6 - protein, 9 aa, Artificial Sequence
  CDR-H3
GTGTYYFDY

SEQ ID NO: 7 - protein, 9 aa, Artificial Sequence
  CDR-L3
LQSNNLPLT

SEQ ID NO: 8 - protein, 5 aa, Artificial Sequence
  CDR-H2
TYSGY

SEQ ID NO: 9 - protein, 9 aa, Artificial Sequence
  CDR-H3
GTGTYYFDH

SEQ ID NO: 10 - protein, 17 aa, Artificial Sequence
  CDR-L1
KSSQSLLYSGNQKNYLA

SEQ ID NO: 11 - protein, 7 aa, Artificial Sequence
  CDR-L2
WASTRDS

SEQ ID NO: 12 - protein, 9 aa, Artificial Sequence
  CDR-L3
QQYSSYPWT

SEQ ID NO: 13 - protein, 7 aa, Artificial Sequence
  CDR-H1
GYSFTGY

SEQ ID NO: 14 - protein, 6 aa, Artificial Sequence
  CDR-H2
NPYSGD

SEQ ID NO: 15 - protein, 9 aa, Artificial Sequence
  CDR-H3
RGDAVPFAY

SEQ ID NO: 16 - protein, 11 aa, Artificial Sequence
  CDR-L1
ITSTDIDEDMN

SEQ ID NO: 17 - protein, 7 aa, Artificial Sequence
  CDR-L2
EGNTLRP

SEQ ID NO: 18 - protein, 9 aa, Artificial Sequence
  CDR-L3
LQSNNMPLT

SEQ ID NO: 19 - protein, 8 aa, Artificial Sequence
  CDR-H1
AYSITSDY

SEQ ID NO: 20 - protein, 5 aa, Artificial Sequence
  CDR-H2
SYSGF

SEQ ID NO: 21 - protein, 9 aa, Artificial Sequence
  CDR-H3
GEITYYFDY

SEQ ID NO: 22 - protein, 7 aa, Artificial Sequence
  CDR-L2
EGNSLRP

SEQ ID NO: 23 - protein, 9 aa, Artificial Sequence
  CDR-H3
GRGTYYFDF

SEQ ID NO: 24 - protein, 107 aa, Artificial Sequence
  ROR1-1 VL
ETTVTQSPASLSMAIGEKVTIRCITSTDIDDDMNWYQQKPGEPPKLLISEGNALRPGVPSRFSSSGYGTDFVFAIENMLSEDVADYYCLQSNKLPLTFGAGTKLELK

SEQ ID NO: 25 - protein, 118 aa, Artificial Sequence
  ROR1-1 VH
EVHLVESGPGLVKPSQSLSLTCTVTGYSITSDYAWNWIRQFPGNRLEWMGYISYSGYTRYNPSLKSRISITRDTSKNQFFLQLNSVTTEDTATYYCAKGTGTYYFDYWGQGTTLTVSS

SEQ ID NO: 26 - protein, 240 aa, Artificial Sequence
  ROR1-1 scFv
ETTVTQSPASLSMAIGEKVTIRCITSTDIDDDMNWYQQKPGEPPKLLISEGNALRPGVPSRFSSSGYGTDFVFAIENMLSEDVADYYCLQSNKLPLTFGAGTKLELKGGGGSGGGGSGGGGSEVHLVESGPGLVKPSQSLSLTCTVTGYSITSDYAWNWIRQFPGNRLEWMGYISYSGYTRYNPSLKSRISITRDTSKNQFFLQLNSVTTEDTATYYCAKGTGTYYFDYWGQGTTLTVSS

SEQ ID NO: 27 - protein, 107 aa, Artificial Sequence
  ROR1-2 VL
DILLTQSPPSLSMAIGEKVTIRCITSTDIDDDMNWYQQKPGEPPKLLISEGNALRPGVPSRFSSSGYGTDFVFAIENMLSEDVADYYCLQSNNLPLTFGAGTKLELN

SEQ ID NO: 28 - protein, 118 aa, Artificial Sequence
  ROR1-2 VH
EVHLVESGPGLVKPSQSLSLTCTVTGYSITSDYAWNWIRQFPGNKLEWMGYITYSGYTRYNPSLKSRISITRDTSKNQFFLQLNSVTSEDTATYYCAKGTGTYYFDHWGQGTTLTVSS

SEQ ID NO: 29 - protein, 240 aa, Artificial Sequence
  ROR1-2 scFv
DILLTQSPPSLSMAIGEKVTIRCITSTDIDDDMNWYQQKPGEPPKLLISEGNALRPGVPSRFSSSGYGTDFVFAIENMLSEDVADYYCLQSNNLPLTFGAGTKLELNGGGGSGGGGSGGGGSEVHLVESGPGLVKPSQSLSLTCTVTGYSITSDYAWNWIRQFPGNKLEWMGYITYSGYTRYNPSLKSRISITRDTSKNQFFLQLNSVTSEDTATYYCAKGTGTYYFDHWGQGTTLTVSS

SEQ ID NO: 30 - protein, 113 aa, Artificial Sequence
  ROR1-3 VL
DIVMTQSPSSQPVSVGEKVTMSCKSSQSLLYSGNQKNYLAWYQQKPGQSPKLLIYWASTRDSGVPDRFTGSGSGTDFTLTISSVKAEDLAVYYCQQYSSYPWTFGGGTKLEIK

SEQ ID NO: 31 - protein, 118 aa, Artificial Sequence
  ROR1-3 VH
EVQLQQSGPELMKPGASMKISCKASGYSFTGYTMNWVKQSHGKNLDWIGLINPYSGDTSYNQQFQGKATLTVDKSSSTAYMELLSLTSEDSAVYFCSRRGDAVPFAYWGQGTLVTVSA

SEQ ID NO: 32 - protein, 246 aa, Artificial Sequence
  ROR1-3 scFv
DIVMTQSPSSQPVSVGEKVTMSCKSSQSLLYSGNQKNYLAWYQQKPGQSPKLLIYWASTRDSGVPDRFTGSGSGTDFTLTISSVKAEDLAVYYCQQYSSYPWTFGGGTKLEIKGGGGSGGGGSGGGGSEVQLQQSGPELMKPGASMKISCKASGYSFTGYTMNWVKQSHGKNLDWIGLINPYSGDTSYNQQFQGKATLTVDKSSSTAYMELLSLTSEDSAVYFCSRRGDAVPFAYWGQGTLVTVSA

SEQ ID NO: 33 - protein, 107 aa, Artificial Sequence
  ROR1-4 VL
ETTVTQSPASLSVATGEKVIIRCITSTDIDEDMNWYQQKPGEPPKLLISEGNTLRPGVPSRFSSSGYGTDFVFTIENTLSEDVADYYCLQSNNMPLTFGAGTKLELK

SEQ ID NO: 34 - protein, 118 aa, Artificial Sequence
  ROR1-4 VH
EVQLQQSGPGLVKPSQSLSLTCTVTAYSITSDYAWNWIRQFPGNKLEWMGYISYSGFTRYNPSLKSRISITRDTSKNEFFLQLNSVTTEDTATYYCARGEITYYFDYWGQGTTLTVSS

SEQ ID NO: 35 - protein, 240 aa, Artificial Sequence
  ROR1-4 scFv
ETTVTQSPASLSVATGEKVIIRCITSTDIDEDMNWYQQKPGEPPKLLISEGNTLRPGVPSRFSSSGYGTDFVFTIENTLSEDVADYYCLQSNNMPLTFGAGTKLELKGGGGSGGGGSGGGGSEVQLQQSGPGLVKPSQSLSLTCTVTAYSITSDYAWNWIRQFPGNKLEWMGYISYSGFTRYNPSLKSRISITRDTSKNEFFLQLNSVTTEDTATYYCARGEITYYFDYWGQGTTLTVSS

SEQ ID NO: 36 - protein, 107 aa, Artificial Sequence
  ROR1-5 VL
ETTVTQSPASLSMAIGEKVTIRCITSTDIDDDMNWYQQKPGEPPKLLISEGNSLRPGVPSRFSSSGYGTDFVFTIENMLSEDVADYYCLQSNNLPLTFGGGTKLEIK

SEQ ID NO: 37 - protein, 118 aa, Artificial Sequence
  ROR1-5 VH
EVQLQESGPGLVKPSQSLSLTCTVTGYSITSDYAWNWIRQFPGNKLEWMGYISYSGYTRYNPSLKSRISITRDTSKKQFFLQLNSVTTEDTATYYCARGRGTYYFDFWGQGTTLTVSS

SEQ ID NO: 38 - protein, 240 aa, Artificial Sequence
  ROR1-5 scFv
ETTVTQSPASLSMAIGEKVTIRCITSTDIDDDMNWYQQKPGEPPKLLISEGNSLRPGVPSRFSSSGYGTDFVFTIENMLSEDVADYYCLQSNNLPLTFGGGTKLEIKGGGGSGGGGSGGGGSEVQLQESGPGLVKPSQSLSLTCTVTGYSITSDYAWNWIRQFPGNKLEWMGYISYSGYTRYNPSLKSRISITRDTSKKQFFLQLNSVTTEDTATYYCARGRGTYYFDFWGQGTTLTVSS

SEQ ID NO: 39 - DNA, 720 bp, Artificial Sequence
  ROR1-1 scFv
gaaacaacggtaactcaatccccagccagtctcagtatggcaataggagagaaagtaacaatcagatgtataaccagtaccgatatagacgatgacatgaattggtaccagcagaaaccgggggagccacccaagcttctgatcagtgaggggaatgcactgcgccccggtgtgccatctcgcttcagtagtagcggatacggtaccgatttcgtatttgccatagaaaacatgctctctgaagatgtagcagattattattgtcttcagtctaataagctgcccctgacatttggcgccgggaccaaactcgaacttaaagggggaggtgggtccgggggaggggggtcaggaggaggcggttctgaagtgcatctcgtcgaaagtgggccagggctcgtcaaaccaagtcagtcattgagccttacctgcacagtgaccggctactctattacgtctgattacgcctggaattggattaggcaatttccgggcaacagactggaatggatgggctatattagctattctgggtatactagatacaaccctagcttgaagtctaggatttccatcacgagagacaccagcaagaaccagttcttcttgcagcttaacagcgtaacgacagaagatacagcaacatactattgcgcgaaaggtactggcacgtattatttcgattactgggggcaggggaccactctgactgtgtctagc

SEQ ID NO: 40 - DNA, 720 bp, Artificial Sequence
  ROR1-2 scFv
gatattctcctgacacagtctcctccttcactcagcatggcaatcggagaaaaggtaacgattcggtgtattacatccacggacatagacgatgacatgaattggtatcaacagaaaccgggtgaaccacccaaactgcttatttccgaagggaatgcccttagaccgggtgtaccaagcagattctcctccagcggatatggcaccgattttgtttttgcgatagaaaatatgttgtccgaggacgtggccgactattactgccttcaatcaaataacctcccattgactttcggcgcaggaactaaattggagcttaacggcggtggaggtagcggaggaggtggttccggcggtggaggctccgaggtccatttggtcgagtccggaccgggattggtgaaaccatcacagtcactctcacttacatgcacggttactggctatagtattacatcagattacgcctggaactggatacgccaatttccagggaataaactggaatggatgggttacattacttacagtggttatacacgatacaatcctagtttgaaaagtcgcatttccattacgagagataccagcaaaaatcagttcttcctccaacttaatagcgtgacgagcgaggacactgctacgtactattgtgcaaagggtactggaacctattatttcgaccattggggccaaggcacaaccctcacggtgtctagc

SEQ ID NO: 41 - DNA, 738 bp, Artificial Sequence
  ROR1-3 scFv
gatatagtaatgactcaaagccccagttcccaaccggtttcagttggtgagaaagtgactatgagctgtaagtcttcccaatctcttctttacagcggcaatcaaaagaattatttggcctggtaccaacagaaacctgggcagtcacccaagctgttgatttactgggcctctacgagagactctggagtgcctgatcgctttacgggaagcggtagtggcacagacttcaccttgacaatatccagtgtaaaagcggaggatctggccgtgtactattgccagcaatatagtagttatccatggacttttggcggaggcactaagcttgagataaaagggggaggggggtctggaggaggaggctcagggggcgggggctcagaggtccaactccagcaatcaggcccagagttgatgaaaccaggagcttcaatgaaaataagttgcaaggcttctgggtactctttcacgggatacaccatgaattgggtcaaacaaagtcacggaaaaaacttggattggataggtctcataaatccctactcaggggacacaagttataaccagcagtttcaaggaaaggctaccctcacggtagataaatcatcatccactgcatatatggaattgttgagcttgacaagtgaagattcagccgtgtatttctgttccaggcggggagatgctgtacctttcgcgtactgggggcagggaactcttgtgacggtatctgcg

SEQ ID NO: 42 - DNA, 720 bp, Artificial Sequence
  ROR1-4 scFv
gaaacgacagttacccaaagtccggcttctcttagcgttgcgactggggagaaagtaataattcggtgcatcacaagtaccgacattgacgaagatatgaattggtaccagcagaagcccggcgagcctccgaaacttctgatcagcgagggtaacacactcaggccaggtgtgcccagccgattctctagctctggctatggcaccgatttcgtttttacgattgagaacaccctctctgaagatgtcgccgattattactgcctgcagagcaacaacatgcccttgaccttcggagctggcacgaagctcgaactgaaaggaggtggagggtcaggtgggggaggcagcggcgggggtggttctgaggtacagctgcaacaatcaggccccggtcttgtaaagccgtcacaatccctcagtcttacctgtacagttacagcttattccattacgtcagactatgcgtggaactggatacggcaatttccgggcaataaactggagtggatgggctatatcagttattccggcttcacgcgctacaacccttctctgaagtctaggattagcattacgcgggacaccagcaagaatgaatttttcctgcagcttaatagcgttacaacggaggatactgccacctactattgcgctagaggtgagataacgtactatttcgactactggggtcaaggaacgaccctcaccgtgtctagc

SEQ ID NO: 43 - DNA, 720 bp, Artificial Sequence
  ROR1-5 scFv
gaaacgacggtaacgcaatcaccggcatctctgtctatggccataggtgagaaagtgacaattcggtgcattactagcacggatatagatgacgacatgaactggtaccagcaaaaacccggagaaccccccaaattgttgatttctgaaggcaactcactccggcctggggtcccttcacgctttagctcatccggttatggcacagactttgttttcacgatcgaaaacatgttgagcgaggacgtggcggattattactgccttcagagtaataatcttcctctcactttcggtgggggtactaagctggagataaaaggtggagggggttcagggggcggaggatcaggcggcggagggagcgaggtgcaactgcaagaatcagggcccggtcttgtgaagccgtcccagagtcttagtttgacctgcacagtgacgggatacagtataacttccgattacgcatggaattggatacgccagttcccagggaataaattggaatggatggggtacatctcctatagcggctatacaaggtataacccaagtctcaaatcccgaatttcaattacaagagacacttctaaaaaacagtttttcctccagcttaactccgtgacaaccgaagacaccgctacatactactgtgcgagaggaaggggtacatattatttcgacttttgggggcagggaacaacgctgaccgtgtcaagc

SEQ ID NO: 44 - protein, 25 aa, Artificial Sequence
  CD8alpha transmembrane domain
IYIWAPLAGTCGVLLLSLVITLYCK

SEQ ID NO: 45 - DNA, 75 bp, Artificial Sequence
  CD8alpha transmembrane domain
atctacatctgggcgcccttggccgggacttgtggggtccttctcctgtcactggttatcaccctttactgcaaa

SEQ ID NO: 46 - protein, 27 aa, Artificial Sequence
  CD28 transmembrane domain
FWVLVVVGGVLACYSLLVTVAFIIFWV

SEQ ID NO: 47 - DNA, 81 bp, Artificial Sequence
  CD28 transmembrane domain
ttttgggtcctcgtcgtagttggaggggtacttgcctgttatagcctcctggttaccgtagcatttattatattctgggtg

SEQ ID NO: 48 - protein, 41 aa, Artificial Sequence
  CD28 costimulatory domain
RSKRSRLLHSDYMNMTPRRPGPTRKHYQPYAPPRDFAAYRS

SEQ ID NO: 49 - DNA, 123 bp, Artificial Sequence
  CD28 costimulatory domain
aggagtaagaggagcaggctcctgcacagtgactacatgaacatgactccccgccgccccgggcccacccgcaagcattaccagccctatgccccaccacgcgacttcgcagcctatcgctcc

SEQ ID NO: 50 - protein, 40 aa, Artificial Sequence
  4-1BB costimulatory domain
RGRKKLLYIFKQPFMRPVQTTQEEDGCSCRFPEEEEGGCE

SEQ ID NO: 51 - DNA, 120 bp, Artificial Sequence
  4-1BB costimulatory domain
cggggcagaaagaaactcctgtatatattcaaacaaccatttatgagaccagtacaaactactcaagaggaagatggctgtagctgccgatttccagaagaagaagaaggaggatgtgaa

SEQ ID NO: 52 - protein, 113 aa, Artificial Sequence
  CD3zeta signaling domain
LRVKFSRSADAPAYQQGQNQLYNELNLGRREEYDVLDKRRGRDPEMGGKPRRKNPQEGLYNELQKDKMAEAYSEIGMKGERRRGKGHDGLYQGLSTATKDTYDALHMQALPPR

SEQ ID NO: 53 - DNA, 339 bp, Artificial Sequence
  CD3zeta signaling domain
ctgagagtgaagttcagcaggagcgcagacgcccccgcgtaccagcagggccagaaccagctctataacgagctcaatctaggacgaagagaggagtacgatgttttggacaagagacgtggccgggaccctgagatggggggaaagccgagaaggaagaaccctcaggaaggcctgtacaatgaactgcagaaagataagatggcggaggcctacagtgagattgggatgaaaggcgagcgccggaggggcaaggggcacgatggcctttaccagggtctcagtacagccaccaaggacacctacgacgcccttcacatgcaggccctgccccctcgc

SEQ ID NO: 54 - protein, 114 aa, Artificial Sequence
  CD3zeta signaling domain
LRVKFSRSADAPAYQQGQNQLFNELNLGRREEFDVLDKRRGRDPEMGGKPQRRKNPQEGLYNELQKDKMAEAYSEIGMKGERRRGKGHDGLFQGLSTATKDTFDALHMQALPPR

SEQ ID NO: 55 - DNA, 342 bp, Artificial Sequence
  CD3zeta signaling domain
ctgagagtgaagttcagcaggagcgcagacgcccccgcgtaccagcagggccagaaccagctctttaacgagctcaatctaggacgaagagaggagttcgatgttttggacaagagacgtggccgggaccctgagatggggggaaagccgcagagaaggaagaaccctcaggaaggcctgtacaatgaactgcagaaagataagatggcggaggcctacagtgagattgggatgaaaggcgagcgccggaggggcaaggggcacgatggccttttccagggtctcagtacagccaccaaggacacctttgacgcccttcacatgcaggccctgccccctcgc

SEQ ID NO: 56 - protein, 20 aa, Artificial Sequence
  B2M signal peptide
MSRSVALAVLALLSLSGLEA

SEQ ID NO: 57 - DNA, 60 bp, Artificial Sequence
  B2M signal peptide
atgtcccgctctgttgctttggctgtgctggcccttttgtcccttagcggactggaggcc

SEQ ID NO: 58 - protein, 21 aa, Artificial Sequence
  CD8alpha signal peptide
MALPVTALLLPLALLLHAARP

SEQ ID NO: 59 - DNA, 63 bp, Artificial Sequence
  CD8alpha signal peptide
atggccttaccagtgaccgccttgctcctgccgctggccttgctgctccacgccgccaggccg

SEQ ID NO: 60 - protein, 45 aa, Artificial Sequence
  CD8alpha hinge region
TTTPAPRPPTPAPTIASQPLSLRPEACRPAAGGAVHTRGLDFACD

SEQ ID NO: 61 - DNA, 135 bp, Artificial Sequence
  CD8alpha hinge region
accacgacgccagcgccgcgaccaccaacaccggcgcccaccatcgcgtcgcagcccctgtccctgcgcccagaggcgtgccggccagcggcggggggcgcagtgcacacgagggggctggacttcgcctgtgat

SEQ ID NO: 62 - protein, 39 aa, Artificial Sequence
  CD28 hinge region
IEVMYPPPYLDNEKSNGTIIHVKGKHLCPSPLFPGPSKP

SEQ ID NO: 63 - DNA, 117 bp, Artificial Sequence
  CD28 hinge region
attgaagttatgtatcctcctccttacctagacaatgagaagagcaatggaaccattatccatgtgaaagggaaacacctttgtccaagtcccctatttcccggaccttctaagccc

SEQ ID NO: 64 - protein, 12 aa, Artificial Sequence
  IgG4 hinge region
ESKYGPPCPPCP

SEQ ID NO: 65 - DNA, 36 bp, Artificial Sequence
  IgG4 hinge region
gaaagcaaatacgggccgccgtgtccaccctgtccg

SEQ ID NO: 66 - protein, 18 aa, Artificial Sequence
  linker
GSTSGSGKPGSGEGSTKG

SEQ ID NO: 67 - protein, 15 aa, Artificial Sequence
  linker
GGGGSGGGGSGGGGS

SEQ ID NO: 68 - protein, 107 aa, Artificial Sequence
  6V7 VL
ETTLTQSPATLSVSPGERAILSCITSTDIDEDMNWYQQKPGQPPKLLISEGNTLRPGVPSRFSGSGSGTDFTLTISSLQPEDVATYYCLQSNNMPLTFGAGTKLELK

SEQ ID NO: 69 - protein, 118 aa, Artificial Sequence
  6V7 VH
QVQLQESGPGLVKPSQTLSLTCTVSAYSITSDYAWNWIRQFPGNKLEWIGYISYSGFTRYNPSLKSRISITRDTSKNQFFLKLNFVTTEDTATYYCARGEITYYFDYWGQGTTLTVSS

SEQ ID NO: 70 - protein, 118 aa, Artificial Sequence; identical to SEQ ID NO: 69
  6V7 ScFv

SEQ ID NO: 71 - DNA, 720 bp, Artificial Sequence
  6V7 ScFv
gagactactctgacccagtcaccagcaacactttctgtctcaccaggcgaacgcgccattctctcctgcatcacaagtacggacattgacgaggatatgaactggtatcagcagaagcccggacagccacccaagttgctgatcagcgagggtaatactcttagacctggggtcccttccagattctcaggctcaggatctggcactgacttcacactgacaatttcctccctccaacctgaggacgtggccacatactattgtcttcagtccaacaatatgccccttacgtttggcgccggcaccaagctggaactgaaaggtggtgggggatccggtggaggtggaagtggtggaggtgggagccaggtacagcttcaggaaagcggccctggcctggtgaaaccatcacagactctgtctctgacgtgtactgtgtccgcctatagcatcacaagcgattatgcctggaactggatccgacagtttcccggaaataaactggaatggattggttacatttcctattcaggctttaccaggtacaatcccagtctcaagtcccggatctctatcacaagagacacaagtaagaatcagttctttttgaaattgaatttcgtcacaactgaggacaccgcgacatattactgtgccaggggtgagatcacttattactttgattactggggacaaggcacaactctgacagtttctagc

SEQ ID NO: 72 - protein, 107 aa, Artificial Sequence
  6V8 VL
ETTLTQSPATLSVSPGEKVIIRCITSTDIDEDMNWYQQKPGQPPKLLISEGNTLRPGVPSRFSGSGSGTDFTLTISSLQPEDVATYYCLQSNNMPLTFGAGTKLELK

SEQ ID NO: 73 - protein, 118 aa, Artificial Sequence
  6V8 VH
QVQLQESGPGLVKPSQTLSLTCTVTAYSITSDYAWNWIRQFPGNKLEWMGYISYSGFTRYNPSLKSRISITRDTSKNQFFLKLNFVTTEDTATYYCARGEITYYFDYWGQGTTLTVSS

SEQ ID NO: 74 - protein, 240 aa, Artificial Sequence
  6V8 ScFv
ETTLTQSPATLSVSPGEKVIIRCITSTDIDEDMNWYQQKPGQPPKLLISEGNTLRPGVPSRFSGSGSGTDFTLTISSLQPEDVATYYCLQSNNMPLTFGAGTKLELKGGGGSGGGGSGGGGSQVQLQESGPGLVKPSQTLSLTCTVTAYSITSDYAWNWIRQFPGNKLEWMGYISYSGFTRYNPSLKSRISITRDTSKNQFFLKLNFVTTEDTATYYCARGEITYYFDYWGQGTTLTVSS

SEQ ID NO: 75 - DNA, 720 bp, Artificial Sequence
  6V8 ScFv
gagacaactcttacacaatcccctgctacactcagcgtgagtcccggcgaaaaggttattatccgatgtatcacttctactgacattgacgaagacatgaattggtatcagcagaaaccaggccagcccccaaaactgctgattagtgaagggaacaccctgaggccaggagtaccctctcggttttcaggaagcggctccggcactgattttacattgactatctctagcctgcagccagaggatgtcgccacttattattgtctgcagagcaacaatatgcctctgacttttggtgcggggacaaagctggagttgaagggaggtggaggttctggcggaggaggaagcggtggtggaggatctcaagttcagctccaggagtcaggtcccggactggtcaaaccctcccagactctgtctttgacatgtacggtcacggcctactcaatcacttccgactatgcatggaactggattcgccagttccccggaaacaaactggaatggatgggctacatcagttactctggctttaccagatataacccatcactcaaaagcagaatcagtatcactagggacaccagcaagaaccagttttttctgaagctgaatttcgtgaccaccgaagacaccgctacctattattgtgccaggggagagatcacttattacttcgattactggggccaggggaccaccctcacagtctcatca

SEQ ID NO: 76 - protein, 107 aa, Artificial Sequence; identical to SEQ ID NO: 72
  6V9 VL

SEQ ID NO: 77 - protein, 107 aa, Artificial Sequence; identical to SEQ ID NO: 72
  6V9 VH

SEQ ID NO: 78 - protein, 240 aa, Artificial Sequence
  6V9 ScFv
ETTLTQSPATLSVSPGEKVIIRCITSTDIDEDMNWYQQKPGQPPKLLISEGNTLRPGVPSRFSGSGSGTDFTLTISSLQPEDVATYYCLQSNNMPLTFGAGTKLELKGGGGSGGGGSGGGGSQVQLQESGPGLVKPSQTLSLTCTVSAYSITSDYAWNWIRQFPGNKLEWIGYISYSGFTRYNPSLKSRISITRDTSKNQYYLQLNSVTTEDTATYYCARGEITYYFDYWGQGTTLTVSS

SEQ ID NO: 79 - DNA, 720 bp, Artificial Sequence
  6V9 ScFv
gaaactacactcacccaaagtcctgccactctgagtgtaagtcctggcgagaaagtcataataagatgcattacaagcaccgatattgatgaggacatgaactggtatcaacagaagcccggacagccacctaaacttctcatcagtgagggcaacactttgaggcctggggtccctagtaggttcagtggcagtggatctggtactgatttcaccctcacaatctcttcattgcagccagaggacgtggccacctactactgcctgcagtccaataatatgccactcacttttggggccggcaccaagctggaactcaagggtggaggaggatcaggtggtggtgggagtggaggaggcggaagtcaagtgcagctccaggagtctggcccaggccttgtgaaaccttcccagaccctgtccctgacttgcaccgtgtcagcatattctataacttccgactacgcctggaactggattcgacagtttcccggcaacaagctggagtggatcggttacatctcctacagcgggtttacaaggtacaacccctctttgaagtcaagaattagtatcacacgggatactagcaagaatcagtactatctgcagttgaattctgtaaccacagaagacaccgcaacctattattgcgccaggggagagatcacctactactttgactactggggacagggcactaccctcaccgtcagctca

SEQ ID NO: 80 - protein, 107 aa, Artificial Sequence
  6V10 VL
ETTLTQSPATLSVSPGERAIIRCITSTDIDEDMNWYQQKPGQPPKLLISEGNTLRPGVPSRFSGSGSGTDFTLTISSLQPEDVATYYCLQSNNMPLTFGAGTKLELK

SEQ ID NO: 81 - protein, 118 aa, Artificial Sequence; identical to SEQ ID NO: 73
  6V10 VH

SEQ ID NO: 82 - protein, 240 aa, Artificial Sequence
  6V10 ScFv
ETTLTQSPATLSVSPGERAIIRCITSTDIDEDMNWYQQKPGQPPKLLISEGNTLRPGVPSRFSGSGSGTDFTLTISSLQPEDVATYYCLQSNNMPLTFGAGTKLELKGGGGSGGGGSGGGGSQVQLQESGPGLVKPSQTLSLTCTVTAYSITSDYAWNWIRQFPGNKLEWMGYISYSGFTRYNPSLKSRISITRDTSKNQFFLKLNFVTTEDTATYYCARGEITYYFDYWGQGTTLTVSS

SEQ ID NO: 83 - DNA, 720 bp, Artificial Sequence
  6V10 ScFv
gaaacaactcttacccagagccctgccactcttagtgtgagccctggagaaagagcaatcatcagatgtatcaccagcacagacatagacgaggatatgaactggtatcagcagaagccaggtcagcctcctaagttgctgatctctgaaggaaacacactgagacctggcgtgccaagcagattttcaggatctgggagtggaacggacttcaccctgaccatctcttccttgcagcccgaagatgttgccacctattactgtctccagtcaaataacatgccactcacctttggggccggcacaaagttggagctgaaaggaggcggaggaagtggaggaggcggaagtggaggaggtggctcacaggttcagctgcaggagagcggaccagggctggtaaagccttcacagaccctttctctgacctgtaccgttacagcctactcaattacaagcgattatgcttggaactggatccggcagttccctgggaacaagctggaatggatgggctatatttcttatagcggcttcactcgatataacccatccctcaaaagtcggatctccatcacacgggacacctccaagaatcagttttttctgaaactgaattttgtgaccactgaggataccgccacctactattgcgctaggggggagatcacgtactacttcgattactggggacagggaacaactctcactgtctcatct

SEQ ID NO: 84 - protein, 107 aa, Artificial Sequence; identical to SEQ ID NO: 80
  6V11 VL

SEQ ID NO: 85 - protein, 118 aa, Artificial Sequence
  6V11 VH
QVQLQESGPGLVKPSQTLSLTCTVSAYSITSDYAWNWIRQFPGNKLEWIGYISYSGFTRYNPSLKSRISITRDTSKNQYYLQLNSVTTEDTATYYCARGEITYYFDYWGQGTTLTVSS

SEQ ID NO: 86 - protein, 240 aa, Artificial Sequence
  6V11 ScFv
ETTLTQSPATLSVSPGERAIIRCITSTDIDEDMNWYQQKPGQPPKLLISEGNTLRPGVPSRFSGSGSGTDFTLTISSLQPEDVATYYCLQSNNMPLTFGAGTKLELKGGGGSGGGGSGGGGSQVQLQESGPGLVKPSQTLSLTCTVSAYSITSDYAWNWIRQFPGNKLEWIGYISYSGFTRYNPSLKSRISITRDTSKNQYYLQLNSVTTEDTATYYCARGEITYYFDYWGQGTTLTVSS

SEQ ID NO: 87 - DNA, 720 bp, Artificial Sequence
  6V11 ScFv
gaaacaacgctcactcagtcacctgccactttgagcgttagtccaggagaaagggcaatcattcggtgcataacttctaccgatattgacgaggacatgaactggtatcagcagaaaccaggacagccaccaaaattgcttatctccgagggcaatactctcagaccaggtgtcccctcaagattttcagggtctggcagtggtacagacttcaccttgaccattagttccctgcagccagaagatgtggctacctattattgtctccagtctaacaacatgcccctgacattcggcgctgggacaaaactggagctgaaaggaggcggtggatctggcggaggtggatctggaggagggggatcacaggtgcaactgcaggaaagtggacccggacttgtaaagccctcccagactctgagtctgacttgcacggtgtcagcctacagcattacgtccgactacgcctggaactggattcggcagttccctggtaataagctggagtggatcggttacatatcatactctgggttcactaggtacaacccaagcctcaagtccagaatcagtataacaagagacacttcaaaaaaccagtactaccttcagctcaatagtgtgaccacagaagacaccgccacctattactgcgcaaggggcgaaataacatattacttcgactactggggccaggggactaccttgaccgtaagcagc

SEQ ID NO: 88 - protein, 107 aa, Artificial Sequence
  6V12 VL
ETTLTQSPATLSVSPGEKVIIRCITSTDIDEDMNWYQQKPGQPPKLLISEGNTLRPGVPSRFSSSGSGTDFTLTISSLQPEDVATYYCLQSNNMPLTFGAGTKLELK

SEQ ID NO: 89 - protein, 118 aa, Artificial Sequence; identical to SEQ ID NO: 73
  6V12 VH

SEQ ID NO: 90 - protein, 240 aa, Artificial Sequence
  6V12 ScFv
ETTLTQSPATLSVSPGEKVIIRCITSTDIDEDMNWYQQKPGQPPKLLISEGNTLRPGVPSRFSSSGSGTDFTLTISSLQPEDVATYYCLQSNNMPLTFGAGTKLELKGGGGSGGGGSGGGGSQVQLQESGPGLVKPSQTLSLTCTVTAYSITSDYAWNWIRQFPGNKLEWMGYISYSGFTRYNPSLKSRISITRDTSKNQFFLKLNFVTTEDTATYYCARGEITYYFDYWGQGTTLTVSS

SEQ ID NO: 91 - DNA, 720 bp, Artificial Sequence
  6V12 ScFv
gaaaccacgttgacacaatctcctgctacactgtcagtgagccccggagaaaaagtcatcatccggtgcatcacatccacagacattgacgaggatatgaactggtatcaacagaagcccggacaacctccaaaactgctgatctcagaaggcaacactctcaggcctggcgtcccatctcgctttagctcaagtggctctggaaccgacttcacactgactatttcctccttgcagcctgaagacgtggcgacatactactgcctccaatccaataacatgcccctgacctttggggctggcacaaagctggagcttaaaggtggtggtggatctggtggaggtggatctgggggtgggggaagtcaggtgcaactgcaagagtccgggcctggactggtgaaacccagccaaaccttgagcctgacgtgtacagtgacagcctacagcattacatccgattatgcctggaattggatccgccagtttccaggaaataagttggagtggatgggctacatctcctacagcggttttaccaggtacaacccatccctgaaaagccgcatcagtattaccagagacacttcaaagaaccaatttttcctgaagctgaactttgtcaccacagaggacactgccacttactattgcgcccgcggggagattacttattacttcgactattggggccaagggaccaccctgactgtatcttcc

SEQ ID NO: 92 - protein, 107 aa, Artificial Sequence; identical to SEQ ID NO: 88
  6V13 VL

SEQ ID NO: 93 - protein, 118 aa, Artificial Sequence; identical to SEQ ID NO: 85
  6V13 VH

SEQ ID NO: 94 - protein, 240 aa, Artificial Sequence
  6V13 ScFv
ETTLTQSPATLSVSPGEKVIIRCITSTDIDEDMNWYQQKPGQPPKLLISEGNTLRPGVPSRFSSSGSGTDFTLTISSLQPEDVATYYCLQSNNMPLTFGAGTKLELKGGGGSGGGGSGGGGSQVQLQESGPGLVKPSQTLSLTCTVSAYSITSDYAWNWIRQFPGNKLEWIGYISYSGFTRYNPSLKSRISITRDTSKNQYYLQLNSVTTEDTATYYCARGEITYYFDYWGQGTTLTVSS

SEQ ID NO: 95 - DNA, 720 bp, Artificial Sequence
  6V13 ScFv
gaaacaaccctcacacagtctcccgctacattgtctgtatctccaggcgaaaaggtaatcattagatgcataacatccacagacatcgatgaggacatgaattggtatcagcaaaagcctggacagccccctaaactgctcatttctgagggcaacaccctgcgacctggtgttcctagtcgcttctcctcaagtgggagcggaaccgacttcaccttgaccatctccagcctgcagccagaagacgtagccacttattattgcctgcagagcaacaacatgccactgacctttggggctggaactaagctcgaacttaaaggtgggggaggtagtggtggtggaggctcaggtggcggaggaagtcaggtgcagctccaggaatctggacctggcctggtgaagccatctcagactctgtccttgacctgcacagtgagtgcttactccatcaccagcgattatgcctggaattggatccggcagttccctggcaacaaactcgaatggatcggatacattagttattccgggtttacgagatacaacccaagcctgaagagtaggattagcatcacgagggacactagcaaaaatcagtactacctgcagctgaattctgtaaccacggaggacaccgccacctattactgcgccagaggcgagatcacttattactttgactattggggccaggggaccacactgaccgtgagtagt